European Patent Application EP 4 722 242 A1, published April 8, 2026. Title: anti-synaptotagmin-2 antibody. Applicant: Jiksak Bioengineering, Inc. The sequence listing filed with the application follows.

SEQUENCE LISTING (17 sequences)

SEQ ID NO: 1 - protein, 119 aa, synthetic construct
QVQLKQSGAELVRPGASVKLSCKASGYTFTDYEMHWVKQTPVHGLEWIGALDPGTGDTAYKQKFKGKATLTADKSSSTAYMVLRSLTSEDSAVYYCTRGASYSNYEDYWGQGTSLTVSS

SEQ ID NO: 2 - protein, 113 aa, synthetic construct
DVVMTQTPLTLSVTIGQPASISCKSSQSLLDSDGKTYLNWLLQRPGQSPKRLIYLVSKLDSGVPDRFTGSGSGTDITLRISTETQKMEFIIAGIILIFRTRSEGGPSWKDGLM

SEQ ID NO: 3 - protein, 6 aa, synthetic construct
TDYEMH

SEQ ID NO: 4 - protein, 17 aa, synthetic construct
ALDPGTGDTAYKQKFKG

SEQ ID NO: 5 - protein, 10 aa, synthetic construct
GASYSNYEDY

SEQ ID NO: 6 - protein, 16 aa, synthetic construct
KSSQSLLDSDGKTYLN

SEQ ID NO: 7 - protein, 7 aa, synthetic construct
LVSKLDS

SEQ ID NO: 8 - protein, 9 aa, synthetic construct
FIIAGIILI

SEQ ID NO: 9 - protein, 419 aa, Homo sapiens
MRNIFKRNQEPIVAPATTTATMPIGPVDNSTESGGAGESQEDMFAKLKEKLFNEINKIPLPPWALIAIAVVAGLLLLTCCFCICKKCCCKKKKNKKEKGKGMKNAMNMKDMKGGQDDDDAETGLTEGEGEGEEEKEPENLGKLQFSLDYDFQANQLTVGVLQAAELPALDMGGTSDPYVKVFLLPDKKKKYETKVHRKTLNPAFNETFTFKVPYQELGGKTLVMAIYDFDRFSKHDIIGEVKVPMNTVDLGQPIEEWRDLQGGEKEEPEKLGDICTSLRYVPTAGKLTVCILEAKNLKKMDVGGLSDPYVKIHLMQNGKRLKKKKTTVKKKTLNPYFNESFSFEIPFEQIQKVQVVVTVLDYDKLGKNEAIGKIFVGSNATGTELRHWSDMLANPRRPIAQWHSLKPEEEVDALLGKNK

SEQ ID NO: 10 - protein, 422 aa, Mus musculus
MRNIFKRNQEPNVAPATTTATMPLAPVAPADNSTESTGPGESQEDMFAKLKEKFFNEINKIPLPPWALIAMAVVAGLLLLTCCFCICKKCCCKKKKNKKEKGKGMKNAMNMKDMKGGQDDDDAETGLTEGEGEGEEEKEPENLGKLQFSLDYDFQANQLTVGVLQAAELPALDMGGTSDPYVKVFLLPDKKKKYETKVHRKTLNPAFNETFTFKVPYQELAGKTLVMAIYDFDRFSKHDIIGEVKVPMNTVDLGQPIEEWRDLQGGEKEEPEKLGDICTSLRYVPTAGKLTVCILEAKNLKKMDVGGLSDPYVKIHLMQNGKRLKKKKTTVKKKTLNPYFNESFSFEIPFEQIQKVQVVVTVLDYDKLGKNEAIGKIFVGSNATGTELRHWSDMLANPRRPIAQWHSLKPEEEVDALLGKNK

SEQ ID NO: 11 - protein, 62 aa, Homo sapiens
MRNIFKRNQEPIVAPATTTATMPIGPVDNSTESGGAGESQEDMFAKLKEKLFNEINKIPLPP

SEQ ID NO: 12 - protein, 60 aa, Mus musculus
MRNIFKRNQEPNVAPATTTATMPLAPVAPADNSTESTGPGESQEDMFAKLKEKFFNEINK

SEQ ID NO: 13 - protein, 25 aa, Mus musculus
MRNIFKRNQEPIVAPATTTATMPIG

SEQ ID NO: 14 - protein, 26 aa, synthetic construct
  SITE 26: note = an additional Cysteine residue for binding to the carrier protein
MRNIFKRNQEPIVAPATTTATMPIGC

SEQ ID NO: 15 - protein, 63 aa, synthetic construct
  SITE 63: note = an additional Lysine residue bound to biotin
MRNIFKRNQEPIVAPATTTATMPIGPVDNSTESGGAGESQEDMFAKLKEKLFNEINKIPLPPK

SEQ ID NO: 16 - protein, 66 aa, synthetic construct
  SITE 66: note = an additional Lysine residue bound to biotin
MRNIFKRNQEPNVAPATTTATMPLAPVAPADNSTESTGPGESQEDMFAKLKEKFFNEINKIPLPPK

SEQ ID NO: 17 - protein, 59 aa, synthetic construct
  SITE 59: note = an additional Lysine residue bound to biotin
MVSESHHEALAAPPVTTVATVLPSNATEPASPGEGKEDAFSKLKEKFMNELHKIPLPPK